European Patent Application EP 4 276 115 A1, published November 15, 2023. Title: ANTI-PD-L1/ANTI-CD47 NATURAL ANTIBODY STRUCTURE-LIKE HETERODIMERIC FORM BISPECIFIC ANTIBODY AND PREPARATION THEREOF. Applicant: BEIJING HANMI PHARMACEUTICAL CO., LTD. The sequence listing filed with the application follows.

SEQUENCE LISTING (48 sequences)

SEQ ID NO: 1 - DNA, 321 bp, Artificial Sequence
  light chain variable region
gacatccagatgacccagtccccttcctccctgtccgcctctgtgggcgacagggtgaccatcacctgcaaggcctcccaggatgtgcacaccgccgtggcttggattcagcagaagcccggcaagtcccccaagctgctgatctactccgcctccaaccggtacaccggcgtgcctagcaggttcagcggaagcggcagcggcaccgacttcaccttcaccatctcctccctgcagcctgaggacatcgccacctattactgccagcagcactacatcacccccctgaccttcggccagggcaccaagctggagatcaag

SEQ ID NO: 2 - protein, 107 aa, Artificial Sequence
  light chain variable region
DIQMTQSPSSLSASVGDRVTITCKASQDVHTAVAWIQQKPGKSPKLLIYSASNRYTGVPSRFSGSGSGTDFTFTISSLQPEDIATYYCQQHYITPLTFGQGTKLEIK

SEQ ID NO: 3 - DNA, 321 bp, Artificial Sequence
  light chain constant region
cgtacggtggccgcccccagcgtcttcatttttccaccctctgacgaacagctgaagtcagggacagcttccgtggtctgtctgctgaacaatttttaccccagggaggccaaagtgcagtggaaggtcgataacgctctgcagagcggaaattctcaggagagtgtgacagaacaggactcaaaagattccacttatagcctgtctagtaccctgacactgtccaaggcagactacgaaaagcataaagtgtatgcctgtgaggtcacacatcagggtctgtcaagccccgtcactaagtccttcaaccggggagaatgc

SEQ ID NO: 4 - protein, 107 aa, Artificial Sequence [sequence omitted]

SEQ ID NO: 5 - DNA, 351 bp, Artificial Sequence
  heavy chain variable region
gaagtgcagctggtgcagtccggcgccgaggtgaagaagcctggctcctccgtgaaggtgtcctgcaaggcctccggcttcaacatcgaggacacctacatccactgggtgaggcaggctcccggacagggactggagtggatgggcaggatcgatcccgccaacgccaacaccaagtacgaccccaagttccagggcagggtgaccatcaccgccgataccagcaccaacaccgcctacatggagctgtcctccctgaggtccgaggacacagccgtgtactactgtggcaggggactgggcgcctggtttgcctactggggacagggcaccctggtgaccgtgtcctcc

SEQ ID NO: 6 - protein, 117 aa, Artificial Sequence
  heavy chain constant region
EVQLVQSGAEVKKPGSSVKVSCKASGFNIEDTYIHWVRQAPGQGLEWMGRIDPANANTKYDPKFQGRVTITADTSTNTAYMELSSLRSEDTAVYYCGRGLGAWFAYWGQGTLVTVSS

SEQ ID NO: 7 - DNA, 990 bp, Artificial Sequence
  heavy chain constant region
gctagcacaaaaggaccttccgtgtttccactggcaccctctagtaagagtacttcaggaggaaccgcagcactgggatgtctggtgaaggactacttcccagagcccgtcaccgtgtcttggaacagtggagcactgacctccggggtccatacatttcctgccgtgctgcagtcatccggtctgtatagcctgagctctgtggtcacagtcccaagttcatccctgggcacccagacatacatctgcaacgtgaatcacaaaccttccaatactaaggtcgacaagaaagtggaacccaagtcctgcgataagacccacacatgccctccctgtcctgctcccgaactgctgggaggaccctccgtcttcctgttcccccccaagcccaaagacacactgatgatcagcaggacccctgaagtgacctgcgtggtcgtggacgtgagccacgaggaccccgaggtcaagtttaactggtacgtggacggcgtggaggtccacaacgccaagaccaagcccagggaggagcagtacaacagcacctacagggtcgtgtccgtgctgaccgtgctccaccaagattggctcaacggcaaggagtataagtgcaaagtcagcaacaaggccctccccgcccccatcgagaaaaccatcagcaaggccaagggccaaccgcgggaacctcaagtgtataccctccctcccagccgggatgagctgaccaagaaccaagtctccctcttgtgcctggtcaagggattctacccttccgacattgccgtcgaatgggagagcaatggccagcccgagaacaactacaagacaaccccccccgtcctgcgcagcgacggatccttcttcctgtactccaagctcaccgtggacaagagccggtggcaacagggcaacgtgttctcctgtagcgtgatgcacgaagccctccacaaccactatacccagaagagcctgagcctcagccccggcaaa

SEQ ID NO: 8 - protein, 330 aa, Artificial Sequence
  heavy chain constant region
ASTKGPSVFPLAPSSKSTSGGTAALGCLVKDYFPEPVTVSWNSGALTSGVHTFPAVLQSSGLYSLSSVVTVPSSSLGTQTYICNVNHKPSNTKVDKKVEPKSCDKTHTCPPCPAPELLGGPSVFLFPPKPKDTLMISRTPEVTCVVVDVSHEDPEVKFNWYVDGVEVHNAKTKPREEQYNSTYRVVSVLTVLHQDWLNGKEYKCKVSNKALPAPIEKTISKAKGQPREPQVYTLPPSRDELTKNQVSLLCLVKGFYPSDIAVEWESNGQPENNYKTTPPVLRSDGSFFLYSKLTVDKSRWQQGNVFSCSVMHEALHNHYTQKSLSLSPGK

SEQ ID NO: 9 - DNA, 996 bp, Artificial Sequence
  heavy chain constant region
gctagcacaaaaggaccttccgtgtttccactggcaccctctagtaagagtacttcaggaggaaccgcagcactgggatgtctggtgaaggactacttcccagagcccgtcaccgtgtcttggaacagtggagcactgacctccggggtccatacatttcctgccgtgctgcagtcatccggtctgtatagcctgagctctgtggtcacagtcccaagttcatccctgggcacccagacatacatctgcaacgtgaatcacaaaccttccaatactaaggtcgacaagaaagtggaacccaagtcctgcgataagacccacacatgccctccctgtcctgctcccgaactgctgggaggaccctccgtcttcctgttcccccccaagcccaaagacacactgatgatcagcaggacccctgaagtgacctgcgtggtcgtggacgtgagccacgaggaccccgaggtcaagtttaactggtacgtggacggcgtggaggtccacaacgccaagaccaagcccagggaggagcagtacgccagcacctacagggtcgtgtccgtgctgaccgtgctccaccaagattggctcaacggcaaggagtataagtgcaaagtcagcaacaaggccctccccgcccccatcgagaaaaccatcagcaaggccaagggccaaccgcgggaacctcaagtgtataccctccctcccagccgggatgagctgaccaagaaccaagtctccctcttgtgcctggtcaagggattctacccttccgacattgccgtcgaatgggagagcaatggccagcccgagaacaactacaagacaaccccccccgtcctgcgcagcgacggatccttcttcctgtactccaagctcaccgtggacaagagccggtggcaacagggcaacgtgttctcctgtagcgtgatgcacgaagccctccacaaccactatacccagaagagcctgagcctcagccccggcaaatgatga

SEQ ID NO: 10 - protein, 330 aa, Artificial Sequence
  heavy chain constant region
ASTKGPSVFPLAPSSKSTSGGTAALGCLVKDYFPEPVTVSWNSGALTSGVHTFPAVLQSSGLYSLSSVVTVPSSSLGTQTYICNVNHKPSNTKVDKKVEPKSCDKTHTCPPCPAPELLGGPSVFLFPPKPKDTLMISRTPEVTCVVVDVSHEDPEVKFNWYVDGVEVHNAKTKPREEQYASTYRVVSVLTVLHQDWLNGKEYKCKVSNKALPAPIEKTISKAKGQPREPQVYTLPPSRDELTKNQVSLLCLVKGFYPSDIAVEWESNGQPENNYKTTPPVLRSDGSFFLYSKLTVDKSRWQQGNVFSCSVMHEALHNHYTQKSLSLSPGK

SEQ ID NO: 11 - DNA, 321 bp, Artificial Sequence
  light chain variable region
gacatcgtgatgacccagtcccagaagttcatgtccacctccgtgggcgaccgggtgagcatcacttgtaaggcctcccagaacgtgaggacctccatcgcttggtatcaacagaagtccggccagtcccccaagactttaatctatttagccagcaatcgtcacactggtgtgcccgatcgtttcactggttctggctccggcaccgacttcactttaaccatctccaacgtgcagagcgaggatttagccgactacttctgtttacagcactggaactaccccttcaccttcggctctggcaccaagctggagatcaag

SEQ ID NO: 12 - protein, 107 aa, Artificial Sequence
  light chain variable region
DIVMTQSQKFMSTSVGDRVSITCKASQNVRTSIAWYQQKSGQSPKTLIYLASNRHTGVPDRFTGSGSGTDFTLTISNVQSEDLADYFCLQHWNYPFTFGSGTKLEIK

SEQ ID NO: 13 - DNA, 354 bp, Artificial Sequence
  heavy chain variable region
gaggtgcagctgcaacagtccggcgccgagctggtgaaacccggtgcctccgtgaagctgagctgcaccgcctccggcttcaacatcgaggacatctacatgcactgggtgaagcagaggcccgaacaaggtttagagtggatcggtcgtatcgaccccgctaacgacaacaccaagtatggccccaagctgcaaggtcgtgccaccatcaccgctgacacctcctccaacaccgcttatttacagctgtccggtttaacctccgaggacaccggagtgtactactgcgtgcggcgtattcctaccgatatcatggactactggggacccggaacctccgtgaccgtgtcctcc

SEQ ID NO: 14 - protein, 118 aa, Artificial Sequence
  heavy chain variable region
EVQLQQSGAELVKPGASVKLSCTASGFNIEDIYMHWVKQRPEQGLEWIGRIDPANDNTKYGPKLQGRATITADTSSNTAYLQLSGLTSEDTGVYYCVRRIPTDIMDYWGPGTSVTVSS

SEQ ID NO: 15 - DNA, 990 bp, Artificial Sequence
  heavy chain constant region
gctagcacaaaaggaccttccgtgtttccactggcaccctctagtaagagtacttcaggaggaaccgcagcactgggatgtctggtgaaggactacttcccagagcccgtcaccgtgtcttggaacagtggagcactgacctccggggtccatacatttcctgccgtgctgcagtcatccggtctgtatagcctgagctctgtggtcacagtcccaagttcatccctgggcacccagacatacatctgcaacgtgaatcacaaaccttccaatactaaggtcgacaagaaagtggaacccaagtcctgcgataagacccacacatgccctccctgtcctgctcccgaactgctgggaggaccctccgtcttcctgttcccccccaagcccaaagacacactgatgatcagcaggacccctgaagtgacctgcgtggtcgtggacgtgagccacgaggaccccgaggtcaagtttaactggtacgtggacggcgtggaggtccacaacgccaagaccaagcccagggaggagcagtacgccagcacctacagggtggtcagcgtgctgaccgtgctgcaccaggattggctcaacggcaaggagtacaagtgcaaagtctccaacaaggccctgcccgcccccatcgagaagaccatctccaaggctaagggacagcccagggagccccaagtgtacaccgagcctcccagccgggatgagctgaccaagaaccaagtctccctcacctgcctggtcaagggattctacccttccgacattgccgtcgaatgggagagcaatggccagcccgagaacaactacaagacaaccccccccgtcctggatagcgacggatccttcttcctgctctccgtgctcaccgtcgacaagagcagatggcagcagggcaacgtgttcagctgtagcgtgatgcacgaggccctgcacaaccactacacccagaagagcctgtccctcagccccggcaag

SEQ ID NO: 16 - protein, 330 aa, Artificial Sequence
  heavy chain constant region
ASTKGPSVFPLAPSSKSTSGGTAALGCLVKDYFPEPVTVSWNSGALTSGVHTFPAVLQSSGLYSLSSVVTVPSSSLGTQTYICNVNHKPSNTKVDKKVEPKSCDKTHTCPPCPAPELLGGPSVFLFPPKPKDTLMISRTPEVTCVVVDVSHEDPEVKFNWYVDGVEVHNAKTKPREEQYASTYRVVSVLTVLHQDWLNGKEYKCKVSNKALPAPIEKTISKAKGQPREPQVYTEPPSRDELTKNQVSLTCLVKGFYPSDIAVEWESNGQPENNYKTTPPVLDSDGSFFLLSVLTVDKSRWQQGNVFSCSVMHEALHNHYTQKSLSLSPGK

SEQ ID NO: 17 - DNA, 321 bp, Artificial Sequence
  light chain variable region
gacatcgtgatgacccagtcccagaagttcatgtccacctccgtgggcgaccgggtgagcatcacttgtaaggcctcccagaacgtgaggacctccatcgcttggtatcaacagaagcctggccagtcccccaagactttaatctatttagccagcaatcgtcacactggtgtgcccgatcgtttcactggttctggctccggcaccgacttcactttaaccatctccaacgtgcagagcgaggatttagccgactacttctgtttacagcactggaactaccccttcaccttcggctctggcaccaagctggagatcaag

SEQ ID NO: 18 - protein, 107 aa, Artificial Sequence
  light chain variable region
DIVMTQSQKFMSTSVGDRVSITCKASQNVRTSIAWYQQKPGQSPKTLIYLASNRHTGVPDRFTGSGSGTDFTLTISNVQSEDLADYFCLQHWNYPFTFGSGTKLEIK

SEQ ID NO: 19 - DNA, 354 bp, Artificial Sequence
  heavy chain variable region
gaggtgcagctgcagcagagcggcgctgaactggtgaagcccggtgccagcgtgaagctgtcttgtaccgcctccggcttcaacatcgaggacatctacatgcactgggtgaagcagcggcccgaacaaggtttagagtggatcggtcgtatcgaccccgccaacgacaacaccaagtacggccccaagttccaaggtcgtgccacaatgaccgccgacacctcctccaacaccgcctatctgcagctgtccggtttaacaagcgaggacaccggcgtgtactactgcgtgaggaggatcaccaccgacgtgatggactactggggacaaggcacttccgtgaccgtgagctcc

SEQ ID NO: 20 - protein, 118 aa, Artificial Sequence
  heavy chain variable region
EVQLQQSGAELVKPGASVKLSCTASGFNIEDIYMHWVKQRPEQGLEWIGRIDPANDNTKYGPKFQGRATMTADTSSNTAYLQLSGLTSEDTGVYYCVRRITTDVMDYWGQGTSVTVSS

SEQ ID NO: 21 - DNA, 321 bp, Artificial Sequence
  light chain variable region
gacatccagatgacccagtcccctagctctttatccgcttccgtgggcgatcgtgtgaccatcacttgtaaggcctcccagaatgtgaggaccagcatcgcttggtatcaacagaagcccggcaaggcccccaagcgtttaatctatttagcctccaataggcacaccggcgtgccttctcgttttagcggctccggctccggcacagagttcactttaaccatctccaatttacagcccgaggacttcgccacctactactgtttacagcactggaactaccccttcaccttcggccaaggcactaagctggagatcaag

SEQ ID NO: 22 - protein, 107 aa, Artificial Sequence
  light chain variable region
DIQMTQSPSSLSASVGDRVTITCKASQNVRTSIAWYQQKPGKAPKRLIYLASNRHTGVPSRFSGSGSGTEFTLTISNLQPEDFATYYCLQHWNYPFTFGQGTKLEIK

SEQ ID NO: 23 - DNA, 354 bp, Artificial Sequence
  heavy chain variable region
caagttcagctggtgcagagcggagccgaggtgaagaagcccggctcctccgtgaaggtgtcttgtaaggcctccggcttcaacatcgaggacatctacatgcactgggtgaggcaagctcccggtcaaggtctggagtggatgggtcgtatcgaccccgccaacgacaacaccaagtacggccctaagctgcaaggtcgggtgaccatcacggccgatgagtccaccaacaccgcctacatggagctgtcctctttacggagcgaggataccgccgtgtactactgcgcgcggcgtattcctaccgacatcatggactactggggccaaggtacaaccgtgaccgtgtcctcc

SEQ ID NO: 24 - protein, 118 aa, Artificial Sequence
  heavy chain variable region
QVQLVQSGAEVKKPGSSVKVSCKASGFNIEDIYMHWVRQAPGQGLEWMGRIDPANDNTKYGPKLQGRVTITADESTNTAYMELSSLRSEDTAVYYCARRIPTDIMDYWGQGTTVTVSS

SEQ ID NO: 25 - DNA, 321 bp, Artificial Sequence; identical to SEQ ID NO: 21
  light chain variable region

SEQ ID NO: 26 - protein, 107 aa, Artificial Sequence; identical to SEQ ID NO: 22
  heavy chain variable region

SEQ ID NO: 27 - DNA, 354 bp, Artificial Sequence
  heavy chain variable region
caagttcagctggtgcagagcggagccgaggtgaagaagcccggctcctccgtgaaggtgtcttgtaaggcctccggcttcaacatcgaggacatctacatgcactgggtgaggcaagctcccggtcaaggtctggagtggatgggtcgtatcgaccccgccaacgacaacaccaagtacggccctaagctgcaaggtcgggtgaccatcacggccgatacctccaccagcaccgcctacatggagctgtcctctttacggagcgaggataccgccgtgtactactgcgtgcggcgtattcctaccgacatcatggactactggggccaaggtacaaccgtgaccgtgtcctcc

SEQ ID NO: 28 - protein, 118 aa, Artificial Sequence
  heavy chain variable region
QVQLVQSGAEVKKPGSSVKVSCKASGFNIEDIYMHWVRQAPGQGLEWMGRIDPANDNTKYGPKLQGRVTITADTSTSTAYMELSSLRSEDTAVYYCVRRIPTDIMDYWGQGTTVTVSS

SEQ ID NO: 29 - DNA, 321 bp, Artificial Sequence
  heavy chain variable region
gacatccagatgacccagtcccctagctctttatccgcttccgtgggcgatcgtgtgaccatcacttgtaaggcctcccagaatgtgaggaccagcatcgcttggtatcaacagaagcccggcaaggcccccaagactttaatctatttagcctccaataggcacaccggcgtgccttctcgttttagcggctccggctccggcacagagttcactttaaccatctccaatttacagcccgaggacttcgccacctactactgtttacagcactggaactaccccttcaccttcggccaaggcactaagctggagatcaag

SEQ ID NO: 30 - protein, 107 aa, Artificial Sequence
  light chain variable region
DIQMTQSPSSLSASVGDRVTITCKASQNVRTSIAWYQQKPGKAPKTLIYLASNRHTGVPSRFSGSGSGTEFTLTISNLQPEDFATYYCLQHWNYPFTFGQGTKLEIK

SEQ ID NO: 31 - DNA, 354 bp, Artificial Sequence
  heavy chain variable region
caagttcagctggtgcagagcggagccgaggtgaagaagcccggctcctccgtgaaggtgtcttgtaaggcctccggcttcaacatcgaggacatctacatgcactgggtgaggcaagctcccggtcaaggtctggagtggatgggtcgtatcgaccccgccaacgacaacaccaagtacggccctaagctgcaaggtcgggtgaccatcacggccgatgagtccaccagcaccgcctacatggagctgtcctctttacggagcgaggataccgccgtgtactactgcgtgcggcgtattcctaccgacatcatggactactggggccaaggtacaaccgtgaccgtgtcctcc

SEQ ID NO: 32 - protein, 118 aa, Artificial Sequence
  heavy chain variable region
QVQLVQSGAEVKKPGSSVKVSCKASGFNIEDIYMHWVRQAPGQGLEWMGRIDPANDNTKYGPKLQGRVTITADESTSTAYMELSSLRSEDTAVYYCVRRIPTDIMDYWGQGTTVTVSS

SEQ ID NO: 33 - DNA, 321 bp, Artificial Sequence; identical to SEQ ID NO: 29
  light chain variable region

SEQ ID NO: 34 - protein, 107 aa, Artificial Sequence; identical to SEQ ID NO: 30
  light chain variable region

SEQ ID NO: 35 - DNA, 354 bp, Artificial Sequence
  heavy chain variable region
caagttcagctggtgcagagcggagccgaggtgaagaagcccggctcctccgtgaaggtgtcttgtaaggcctccggcttcaacatcgaggacatctacatgcactgggtgaggcaagctcccggtcaaggtctggagtggatgggtcgtatcgaccccgccaacgacaacaccaagtacggccctaagctgcaaggtcgggtgaccatcacggccgatacctccaccaacaccgcctacatggagctgtcctctttacggagcgaggataccgccgtgtactactgcgtgcggcgtattcctaccgacatcatggactactggggccaaggtacaaccgtgaccgtgtcctcc

SEQ ID NO: 36 - protein, 118 aa, Artificial Sequence
  heavy chain variable region
QVQLVQSGAEVKKPGSSVKVSCKASGFNIEDIYMHWVRQAPGQGLEWMGRIDPANDNTKYGPKLQGRVTITADTSTNTAYMELSSLRSEDTAVYYCVRRIPTDIMDYWGQGTTVTVSS

SEQ ID NO: 37 - protein, 10 aa, Artificial Sequence
  PDL1 HCDR1
GFNIEDTYIH

SEQ ID NO: 38 - protein, 17 aa, Artificial Sequence
  PDL1 HCDR2
RIDPANANTKYDPKFQG

SEQ ID NO: 39 - protein, 8 aa, Artificial Sequence
  PDL1 HCDR3
GLGAWFAY

SEQ ID NO: 40 - protein, 11 aa, Artificial Sequence
  PDL1 LCDR1
KASQDVHTAVA

SEQ ID NO: 41 - protein, 7 aa, Artificial Sequence
  PDL1 LCDR2
SASNRYT

SEQ ID NO: 42 - protein, 9 aa, Artificial Sequence
  PDL1 LCDR3
QQHYITPLT

SEQ ID NO: 43 - protein, 10 aa, Artificial Sequence
  CD47 HCDR1
GFNIEDIYMH

SEQ ID NO: 44 - protein, 17 aa, Artificial Sequence
  CD47 HCDR2
RIDPANDNTKYGPKLQG

SEQ ID NO: 45 - protein, 9 aa, Artificial Sequence
  CD47 HCDR3
RIPTDIMDY

SEQ ID NO: 46 - protein, 11 aa, Artificial Sequence
  CD47 LCDR1
KASQNVRTSIA

SEQ ID NO: 47 - protein, 7 aa, Artificial Sequence
  CD47 LCDR2
LASNRHT

SEQ ID NO: 48 - protein, 9 aa, Artificial Sequence
  CD47 LCDR3
LQHWNYPFT